European Patent Application EP 4 400 111 A1, published July 17, 2024. Title: Gut microbes against infectious diseases and its use. Applicant: SNJ Pharma Inc. The sequence listing filed with the application follows.

SEQUENCE LISTING (4 sequences)

SEQ ID NO: 1 - DNA, 20 bp, synthetic construct
  source 1..20: mol_type = other DNA
agagtttgatcctggctcag

SEQ ID NO: 2 - DNA, 19 bp, synthetic construct
  source 1..19: mol_type = other DNA
ggttaccttgttacgactt

SEQ ID NO: 3 - DNA, 1408 bp, Oribacterium sp.
  source 1..1408: mol_type = other DNA
tgcaagtcgaacgagatgcgttattggaaagcttcggccggaagatgcgttatctagtggcggacgggtgagtaacacgtgggtaacctgccttatggagggggataacagagagaaatcactgctaataccgcataagcacacagtaccgcatggcagagtgtgaaaagatttatcgccataagatggacccgcgtctgattagccagttggcagggtaaaagcctaccaaagcaacgatcagtagccgatctgagaggatgaccggccacattgggactgagacacggcccaaactcctacgggaggcagcagtggggaatattgcacaatgggggaaaccctgatgcagcgaacgccgcgtgagtgaagaagtatttcggtatgtaaagctctatcagcagggaagataatgacagtacctgactaagaagccccggctaactacgtgccagcagccgcggtaatacgtagggggcaagcgttatccggatttactgggtgtaaagggagcgtagacggagtggcaagtctgaagtgaaaaccctgggcttaacctggggactgctttggaaactgttaatctagagtgttggagaggtaagtggaattcctggtgtagcggtgaaatgcgtagatatcaggaagaacaccggaggcgaaggcggcttactggacaataactgacgttgaggctcgaaagcgtggggatcaaacaggattagataccctggtagtccacgctgtaaacgatgaatactaggtgtcgggggagcaaagcttctcggtgccgtcgctaacgcaataagtattccacctggggagtacgttcgcaagaatgaaactcaaaggaattgacggggacccgcacaagcggtggagcatgtggtttaattcgaagcaacgcgaagaaccttaccaagtcttgagatcccattgacagagtgtgtaatgcattttcccttcggggcaatgggtgacaggtggtgcatggttgtcgtcagctcgtgtcgtgagatgttgggattaagttcccgcaacgagcgcaacccctatagttagtagtccagcagtaagatgggacactctaactagactgccagggataacctggaggaaggcggggatgacgtcaaatcatcatgccccttatgacttgggctacacacgtgctacaatggcgtaaacaaagggaagcaagagggtgaccttaagcaaatctcaaaaataacgtctcagttcggactgtagtctgcaacccgactacacgaagctggaatcgctagtaatcgcagatcagcatgctgcggtgaatacgttcccgggtcttgtacacaccgcccgtcacaccatgggagttggtaatgcccgaagtcagtgtcccaagagagggagctgccgaaggcag

SEQ ID NO: 4 - DNA, 1417 bp, Ruminococcus gnavus
  source 1..1417: mol_type = other DNA
ccttcggcagctccctccttgcggttgggtcactgacttcgggcgttactgactcccatggtgtgacgggcggtgtgtacaagacccgggaacgtattcaccgcgacattctgattcgcgattactagcgattccagcttcatgtagtcgagttgcagactacaatccgaactgagacgttatttttgggatttgctccccctcgcgggctcgcttccctttgtttacgccattgtagcacgtgtgtagccctggtcataaggggcatgatgatttgacgtcatccccaccttcctccaggttatccctggcagtctctctagagtgcccatccaaaatgctggctactaaagataggggttgcgctcgttgcgggacttaacccaacatctcacgacacgagctgacgacaaccatgcaccacctgtctcctctgtcccgaaggaaagctccgattaaagagcggtcagagggatgtcaagaccaggtaaggttcttcgcgttgcttcgaattaaaccacatgctccaccgcttgtgcgggtccccgtcaattcctttgagtttcattcttgcgaacgtactccccaggtggaatacttattgcgtttgctgcggcaccgaatggctttgccacccgacacctagtattcatcgtttacggcgtggactaccagggtatctaatcctgtttgctccccacgctttcgagccctcaacgtcagtcatcgtccagaaagccgccttcgccactggtgttcctcctaatatctacgcatttcaccgctacactaggaattccgctttcctctccgacactctagcctgacagttccaaatgcagtcccggggttgagccccgggctttcacatctggcttgccatgccgtctacgctccctttacacccagtaaatccggataacgcttgccccctacgtattaccgcggctgctggcacgtagttagccggggcttcttagtcaggtaccgtcattttcttccctgctgatagagctttacataccgaaatacttcatcgctcacgcggcgtcgctgcatcagggtttcccccattgtgcaatattccccactgctgcctcccgtaggagtttgggccgtgtctcagtcccaatgtggccggtcaccctctcaggtcggctactgatcgtcggcttggtaggccgttaccccagccaactacctaatcagacgcgggtccatctcataccaccggagtttttcacaccgtaccatgcggtactgtgcgcttatgcggtattagcagccgtttccaactgttatccccctgtatgaggcaggttacccacgcgttactcacccgtccgccgctcagtcaccaaggcttcaatccgaagaaatccgtcaaggtgcttcgctcgacttgcatgggttaagc